European Patent Application EP 4 289 968 A1, published December 13, 2023. Title: PRIMER PROBE SET AND KIT FOR RT-PCR DETECTION OF HUMAN LEUKOTRIENE RECEPTOR CYSLTR1 MRNA. Applicant: HANGZHOU ZHEDA DIXUN BIOLOGICAL GENE ENGINEERING CO., LTD. The sequence listing filed with the application follows.

SEQUENCE LISTING (9 sequences)

SEQ ID NO: 1 - DNA, 21 bp, Artificial Sequence
  Primer CysLTR1-F
aacctatcacaagaagtcagc

SEQ ID NO: 2 - DNA, 20 bp, Artificial Sequence
  Primer CysLTR1-R
ccaaagagccaaatgccttt

SEQ ID NO: 3 - DNA, 20 bp, Artificial Sequence
  Probe C1-Probe
cactgcctctccgtgtggtc

SEQ ID NO: 4 - DNA, 21 bp, Artificial Sequence
  Primer GAPDH-F
gacaacagcctcaagatcatc

SEQ ID NO: 5 - DNA, 18 bp, Artificial Sequence
  Primer GAPDH-R
cgccacagtttcccggag

SEQ ID NO: 6 - DNA, 24 bp, Artificial Sequence
  Probe G-Probe
actcatgaccacagtccatgccat

SEQ ID NO: 7 - DNA, 19 bp, Artificial Sequence
  Primer CysLTR1-F
gtatcttctgccacatgcc

SEQ ID NO: 8 - DNA, 21 bp, Artificial Sequence
  Primer CysLTR1-R
ttgccaaagaagcctacaaca

SEQ ID NO: 9 - DNA, 22 bp, Artificial Sequence
  Probe C1-Probe
ccgcaatcaagtgtattccacc